European Patent Application EP 4 570 819 A9, published September 23, 2026. Title: LONG-ACTING DUAL-AGONIST COMPOUND. Applicant: CHENGDU AODA BIOTECHNOLOGY CO., LTD. The sequence listing filed with the application follows.

SEQUENCE LISTING (5 sequences)

SEQ ID NO: 1 - protein, 39 aa, synthetic construct
  MOD_RES 2..20: note; note (original language) = The 20th position X is a lysine modified with AEEA-AEEA-γGlu-20 alkyl diacid.; note; note (original language) = X at second position is Aib.
HXQGTFTSDYSKYLDEKKAXEFVEWLLEGGPSSGAPPPS

SEQ ID NO: 2 - protein, 39 aa, synthetic construct; identical to SEQ ID NO: 1
  MOD_RES 2..20: note; note (original language) = The 20th position X is a lysine modified with PEG5CH2CO-γGlu-20 alkyl diacid.; note; note (original language) = X at second position is Aib

SEQ ID NO: 3 - protein, 39 aa, synthetic construct; identical to SEQ ID NO: 1
  MOD_RES 2..20: note; note (original language) = X at second position is Aib; note; note (original language) = The 20th position X is a lysine modified with Gly-Gly-Ser-Gly-Ser-Gly-γGlu-20 alkyl diacid-γGlu-20 alkyl diacid.

SEQ ID NO: 4 - protein, 39 aa, synthetic construct; identical to SEQ ID NO: 1
  MOD_RES 2..20: note; note (original language) = X at second position is Aib; note; note (original language) = The 20th position X is a lysine modified with Gly-Gly-Glu-Gly-Glu-Gly-γGlu-20 alkyl diacid.

SEQ ID NO: 5 - protein, 34 aa, synthetic construct
  MOD_RES 2..20: note; note (original language) = The 20th position X is a lysine modified with AEEA-AEEA-γGlu-20 alkyl diacid.; note; note (original language) = X at second position is Aib
HXQGTFTSDYSKYLDEKKAXEFVEWLLEGGPSSG